European Patent Specification EP 4 126 049 B1, published August 20, 2025. Title: Fast-track humanisation. Applicant: Elasmogen Ltd. The sequence listing filed with the application follows.

SEQUENCE LISTING (101 sequences)

SEQ ID NO: 1 - protein, 28 aa, artificial sequence
  Consensus sequence - humanised FW1
  misc_feature (1)..(1): Where X is - or D
  misc_feature (2)..(2): Where X is A or I or T
  misc_feature (3)..(3): Where X is S or Q or R
  misc_feature (4)..(4): Where X is V or M
  misc_feature (5)..(5): Where X is N or T or D
  misc_feature (25)..(25): Where X is L or V
  misc_feature (26)..(26): Where X is T or R
  misc_feature (27)..(27): Where X is D or G
  misc_feature (28)..(28): Where X is T or A or S
XXXXXQSPSSLSASVGDRVTITCVXXXX

SEQ ID NO: 2 - protein, 10 aa, artificial sequence
  Consensus sequence - FW2
  misc_feature (2)..(2): Where X is S or Y
  misc_feature (4)..(4): Where X is F or Y
  misc_feature (5)..(5): Where X is R or Q
  misc_feature (6)..(6): Where X is K or Q
  misc_feature (7)..(7): Where X is N or K
  misc_feature (8)..(8): Where X is P or S
  misc_feature (10)..(10): Where X is T or S
TXWXXXXXGX

SEQ ID NO: 3 - protein, 8 aa, artificial sequence
  Consensus sequence - FW3a
  misc_feature (3)..(3): Where X is Y or F
  misc_feature (4)..(4): Where X is V or S
  misc_feature (5)..(5): Where X is E or G
  misc_feature (6)..(6): Where X is S or T
  misc_feature (7)..(7): Where X is V or G or I
  misc_feature (8)..(8): Where X is N or S
GRXXXXXX

SEQ ID NO: 4 - protein, 20 aa, artificial sequence
  Consensus sequence - FW3b
  misc_feature (2)..(2): Where X is S or T
  misc_feature (4)..(4): Where X is R or T
  misc_feature (6)..(6): Where X is K or S or N
  misc_feature (7)..(7): Where X is D or S
  misc_feature (9)..(9): Where X is T or Q
  misc_feature (10)..(10): Where X is V or P
  misc_feature (11)..(11): Where X is A or E
  misc_feature (13)..(13): Where X is S or F
  misc_feature (14)..(14): Where X is A or G
  misc_feature (17)..(17): Where X is Y or R or I
  misc_feature (19)..(19): Where X is K or R or A
  misc_feature (20)..(20): Where X is A or S or L
FXLXIXXLXXXDXXTYXCXX

SEQ ID NO: 5 - protein, 10 aa, artificial sequence
  Consensus sequence - FW4
  misc_feature (1)..(1): Where X is D or Y or F
  misc_feature (3)..(3): Where X is A or G or Q
  misc_feature (6)..(6): Where X is K or V
  misc_feature (7)..(7): Where X is V or L
  misc_feature (8)..(8): Where X is E or T
  misc_feature (9)..(9): Where X is I or V
  misc_feature (10)..(10): Where X is K or N
XGXGTXXXXX

SEQ ID NO: 6 - protein, 27 aa, artificial sequence
  Consensus sequence - V1 to V5 FW1
  misc_feature (1)..(1): Where X is A or T
  misc_feature (2)..(2): Where X is S or R
  misc_feature (4)..(4): Where X is N or D
  misc_feature (24)..(24): Where X is L or V
  misc_feature (26)..(26): Where X is D or G
  misc_feature (27)..(27): Where X is T or A
XXVXQSPSSLSASVGDRVTITCVXTXX

SEQ ID NO: 7 - protein, 28 aa, artificial sequence
  Consensus sequence - V6 FW1
  misc_feature (25)..(25): Where X is L or V
  misc_feature (27)..(27): Where X is D or G
  misc_feature (28)..(28): Where X is T or A
DIQMTQSPSSLSASVGDRVTITCVXTXX

SEQ ID NO: 8 - protein, 27 aa, artificial sequence
  soloMER D1v2 / C4v1 QuadX - FW1
ARVDQSPSSLSASVGDRVTITCVLRDS

SEQ ID NO: 9 - protein, 10 aa, artificial sequence
  Consensus sequence - V1 to V3 FW2
  misc_feature (2)..(2): Where X is S or Y
  misc_feature (4)..(4): Where X is F or Y
  misc_feature (10)..(10): Where X is T or S
TXWXRKNPGX

SEQ ID NO: 10 - protein, 10 aa, artificial sequence
  Consensus sequence - V4 to V6 FW2
  misc_feature (2)..(2): Where X is S or Y
  misc_feature (4)..(4): Where X is Y or F
  misc_feature (10)..(10): Where X is T or S
TXWXQQKPGX

SEQ ID NO: 11 - protein, 10 aa, artificial sequence
  soloMER D1v2 / C4v1 QuadX - FW2
TYWYRKKSGS

SEQ ID NO: 12 - protein, 8 aa, artificial sequence
  FW3a V1, V2, V3
GRYVESVN

SEQ ID NO: 13 - protein, 8 aa, artificial sequence
  FW3a V4, V5, V6
GRFSGSGS

SEQ ID NO: 14 - protein, 8 aa, artificial sequence
  soloMER D1v2 FW3a
GRYVETVN

SEQ ID NO: 15 - protein, 8 aa, artificial sequence
  soloMER C4v1 FW3a
GRYVETIN

SEQ ID NO: 16 - protein, 20 aa, artificial sequence
  Consensus sequence - FW3b
  misc_feature (17)..(17): Where X is Y or I
  misc_feature (19)..(19): Where X is K or R
FSLRIKDLTVADSATYXCXA

SEQ ID NO: 17 - protein, 20 aa, artificial sequence
  Consensus sequence - FW3b
  misc_feature (17)..(17): Where X is Y or I
  misc_feature (19)..(19): Where X is K or R
FTLTISSLQPEDFATYXCXA

SEQ ID NO: 18 - protein, 20 aa, artificial sequence
  soloMER D1v2 FW3b
FTLTISSLQPEDFATYYCAS

SEQ ID NO: 19 - protein, 20 aa, artificial sequence
  soloMER C4v1 Fw3b
FSLRINDLTVEDSGTYRCKL

SEQ ID NO: 20 - protein, 10 aa, artificial sequence
  Consensus sequence - FW4
  misc_feature (1)..(1): Where X is D or Y or F
  misc_feature (3)..(3): Where X is A or G or Q
  misc_feature (7)..(7): Where X is V or L
XGXGTKXEIK

SEQ ID NO: 21 - protein, 10 aa, artificial sequence
  soloMER D1v2 / C4v1 QuadX - FW4
YGGGTVVTVN

SEQ ID NO: 22 - protein, 10 aa, artificial sequence
  Consensus sequence - FW2
  misc_feature (2)..(2): Where X is S or Y
  misc_feature (4)..(4): Where X is F or Y
  misc_feature (5)..(5): Where X is R or Q
  misc_feature (6)..(6): Where X is K or Q
  misc_feature (7)..(7): Where X is N or K
  misc_feature (8)..(8): Where X is P or S
  misc_feature (10)..(10): Where X is T or S
TXWXXXXXGX

SEQ ID NO: 23 - protein, 8 aa, artificial sequence
  Consensus sequence - FW3a
  misc_feature (3)..(3): Where X is Y or F
  misc_feature (4)..(4): Where X is V or S
  misc_feature (5)..(5): Where X is E or G
  misc_feature (6)..(6): Where X is S or T
  misc_feature (7)..(7): Where X is V or G or I
  misc_feature (8)..(8): Where X is N or S
GRXXXXXX

SEQ ID NO: 24 - protein, 20 aa, artificial sequence
  Consensus sequence - FW3b
  msic_feature (2)..(2): Where X is S or T
  msic_feature (4)..(4): Where X is R or T
  msic_feature (6)..(6): Where X is K or S or N
  msic_feature (7)..(7): Where X is D or S
  msic_feature (9)..(9): Where X is T or Q
  msic_feature (10)..(10): Where X is V or P
  msic_feature (11)..(11): Where X is A or E
  msic_feature (13)..(13): Where X is S or F
  msic_feature (14)..(14): Where X is A or G
  msic_feature (17)..(17): Where X is Y or R or I
  msic_feature (19)..(19): Where X is K or R or A
  msic_feature (20)..(20): Where X is A or S or L
FXLXIXXLXXXDXXTYXCXX

SEQ ID NO: 25 - protein, 10 aa, artificial sequence
  Consensus sequence - FW4
  misc_feature (1)..(1): Where X is D or Y
XGAGTKVEIK

SEQ ID NO: 26 - protein, 6 aa, artificial sequence
  Consensus sequence - CDR1
  misc_feature (1)..(1): Where X is Y or T or R or I or K or N or S
  misc_feature (2)..(2): Where X is C or Y
  misc_feature (3)..(3): Where X is P or S or A or G
  misc_feature (4)..(4): Where X is W or L
  misc_feature (5)..(5): Where X is H or S or Y
  misc_feature (6)..(6): Where X is N or R or G or S
XXXXXX

SEQ ID NO: 27 - protein, 9 aa, artificial sequence
  Consensus sequence - HV2
  misc_feature (1)..(1): Where X is S or T or P
  misc_feature (2)..(2): Where X is N or D
  misc_feature (3)..(3): Where X is Q or W
  misc_feature (6)..(6): Where X is I or M
  misc_feature (9)..(9): Where X is G or S
XXXERXSIX

SEQ ID NO: 28 - protein, 5 aa, artificial sequence
  Consensus sequence - HV4
  misc_feature (2)..(2): Where X is G or R
  misc_feature (3)..(3): Where X is T or P or S
  misc_feature (4)..(4): Where X is K or M
KXXXS

SEQ ID NO: 29 - protein, 6 aa, artificial sequence
  CDR1 of the first VNAR domain
HCATSS

SEQ ID NO: 30 - protein, 6 aa, artificial sequence
  CDR1 of the second VNAR domain
NCGLSS

SEQ ID NO: 31 - protein, 6 aa, artificial sequence
  CDR1 of the VNAR domain
NCALSS

SEQ ID NO: 32 - protein, 9 aa, artificial sequence
  HV2 of the first and second VNAR domain
TNEESISKG

SEQ ID NO: 33 - protein, 5 aa, artificial sequence
  HV4 of the first VNAR domain
SGSKS

SEQ ID NO: 34 - protein, 5 aa, artificial sequence
  HV4 of the second VNAR domain
EGSKS

SEQ ID NO: 35 - protein, 11 aa, artificial sequence
  CDR3 of the first VNAR domain
ECQYGLAEYDV

SEQ ID NO: 36 - protein, 14 aa, artificial sequence
  CDR3 of the second VNAR domain
SWWTQNWRCSNSDV

SEQ ID NO: 37 - protein, 23 aa, artificial sequence
  CDR3 of a further VNAR domain
YIPCIDELVYMISGGTSGPIHDV

SEQ ID NO: 38 - protein, 106 aa, artificial sequence
  soloMER D1 QuadX v2
ARVDQSPSSLSASVGDRVTITCVLRDSHCATSSTYWYRKKSGSTNEESISKGGRYVETVNSGSKSFTLTISSLQPEDFATYYCASECQYGLAEYDVYGGGTVVTVN

SEQ ID NO: 39 - protein, 109 aa, artificial sequence
  soloMER DC4 QuadX v2
ARVDQSPSSLSASVGDRVTITCVLRDSNCGLSSTYWYRKKSGSTNEESISKGGRYVETINEGSKSFSLRINDLTVEDSGTYRCKLSWWTQNWRCSNSDVYGGGTVVTVN

SEQ ID NO: 40 - protein, 107 aa, artificial sequence
  DPK-9
DIQMTQSPSSLSASVGDRVTITCRASQSISSYLNWYQQKPGKAPKLLIYAASSLQSGVPSRFSGSGSGTDFTLTISSLQPEDFATYYCQQSYSTPNTFGQGTKVEIK

SEQ ID NO: 41 - DNA, 19 bp, artificial sequence
  Primer D3_FOR_NCoI
agccggccatggccgcttc

SEQ ID NO: 42 - DNA, 24 bp, artificial sequence
  Primer D3_REV_NotI
atgtgcggccgcccctgaggcctg

SEQ ID NO: 43 - protein, 106 aa, artificial sequence
  D1
ARVDQTPQTITKETGESLTINCVLRDSHCATSSTYWYRKKSGSTNEESISKGGRYVETVNSGSKSFSLRINDLTVEDSGTYRCASECQYGLAEYDVYGGGTVVTVN

SEQ ID NO: 44 - protein, 106 aa, artificial sequence
  D1-V1
ARVDQSPSSLSASVGDRVTITCVLRDSHCATSSTYWYRKKSGSTNEESISKGGRYVETVNSGSKSFSLRINDLTVEDSGTYRCASECQYGLAEYDVYGGGTKVEIK

SEQ ID NO: 45 - protein, 106 aa, artificial sequence
  D1-V2
ARVDQSPSSLSASVGDRVTITCVLRDSHCATSSTYWYRKKSGSTNEESISKGGRYVETVNSGSKSFTLTISSLQPEDFATYYCASECQYGLAEYDVYGGGTKVEIK

SEQ ID NO: 46 - protein, 106 aa, artificial sequence
  D1-V3
ARVDQSPSSLSASVGDRVTITCVLRDSHCATSSTYWYRKKPGSTNEESISKGGRFSGSGSSGSKSFTLTISSLQPEDFATYYCASECQYGLAEYDVFGQGTKVEIK

SEQ ID NO: 47 - protein, 106 aa, artificial sequence; identical to SEQ ID NO: 46
  D1-V4

SEQ ID NO: 48 - protein, 106 aa, artificial sequence
  D1-V5
ARVDQSPSSLSASVGDRVTITCVLRDSHCATSSTYWYQQKPGSTNEESISKGGRFSGSGSSGSKSFTLTISSLQPEDFATYYCASECQYGLAEYDVFGQGTKVEIK

SEQ ID NO: 49 - protein, 107 aa, artificial sequence
  D1-V6
DIQMTQSPSSLSASVGDRVTITCVLRDSHCATSSTYWYQQKPGSTNEESISKGGRFSGSGSSGSKSFTLTISSLQPEDFATYYCASECQYGLAEYDVFGQGTKVEIK

SEQ ID NO: 50 - protein, 109 aa, artificial sequence
  C4
ARVDQTPQTITKETGESLTINCVLRDSNCGLSSTYWYRKKSGSTNEESISKGGRYVETINEGSKSFSLRINDLTVEDSGTYRCKLSWWTQNWRCSNSDVYGGGTVVTVN

SEQ ID NO: 51 - protein, 109 aa, artificial sequence
  C4-V1
ARVDQSPSSLSASVGDRVTITCVLRDSNCGLSSTYWYRKKSGSTNEESISKGGRYVETINEGSKSFSLRINDLTVEDSGTYRCKLSWWTQNWRCSNSDVYGGGTKVEIK

SEQ ID NO: 52 - protein, 109 aa, artificial sequence
  C4-V2
ARVDQSPSSLSASVGDRVTITCVLRDSNCGLSSTYWYRKKSGSTNEESISKGGRYVETINEGSKSFTLTISSLQPEDFATYYCKLSWWTQNWRCSNSDVFGQGTKVEIK

SEQ ID NO: 53 - protein, 109 aa, artificial sequence
  C4-V3
ARVDQSPSSLSASVGDRVTITCVLRDSNCGLSSTYWYQQKPGKTNEESISKGGRYVETINEGSKSFTLTISSLQPEDFATYYCKLSWWTQNWRCSNSDVFGQGTKVEIK

SEQ ID NO: 54 - protein, 109 aa, artificial sequence
  C4-V4
ARVDQSPSSLSASVGDRVTITCVLRDSNCGLSSTYWYRKKSGSTNEESISKGGRFSGSGSEGSKSFTLTISSLQPEDFATYYCKLSWWTQNWRCSNSDVFGQGTKVEIK

SEQ ID NO: 55 - protein, 109 aa, artificial sequence
  C4-V5
ARVDQSPSSLSASVGDRVTITCVLRDSNCGLSSTYWYQQKPGSTNEESISKGGRFSGSGSEGSKSFTLTISSLQPEDFATYYCKLSWWTQNWRCSNSDVFGQGTKVEIK

SEQ ID NO: 56 - protein, 110 aa, artificial sequence
  C4-V6
DIQMTQSPSSLSASVGDRVTITCVLRDSNCGLSSTYWYQQKPGSTNEESISKGGRFSGSGSEGSKSFTLTISSLQPEDFATYYCKLSWWTQNWRCSNSDVFGQGTKVEIK

SEQ ID NO: 57 - protein, 140 aa, artificial sequence
  Consensus
ARVDQTPQTITKETGESLTINCVLRDSHCATSSTYWYRKKSGSTNEESISKGGRYVETVNSGSKSFTLTISSLQPEDFATYYCASECQYGLAEYDVYGGGTVVTVNGSGGGSGGGGSGEPKSSDKTHTCPPCPAPELLGG

SEQ ID NO: 58 - protein, 484 aa, artificial sequence
  soloMER D1-Fc-C4 Quad-X (NAR FW1)
ARVDQTPQTITKETGESLTINCVLRDSHCATSSTYWYRKKSGSTNEESISKGGRYVETVNSGSKSFTLTISSLQPEDFATYYCASECQYGLAEYDVYGGGTKVEIKGSGGGSGGGGSGEPKSSDKTHTCPPCPAPELLGGPSVFLFPPKPKDTLMISRTPEVTCVVVDVSHEDPEVKFNWYVDGVEVHNAKTKPREEQYNSTYRVVSVLTVLHQDWLNGKEYKCKVSNKALPAPIEKTISKAKGQPREPQVYTLPPSRDELTKNQVSLTCLVKGFYPSDIAVEWESNGQPENNYKTTPPVLDSDGSFFLYSKLTVDKSRWQQGNVFSCSVMHEALHNHYTQKSLSLSPGKGGGGSGGGGSGGGGSGGGGSGGGGSARVDQTPQTITKETGESLTINCVLRDSNCGLSSTYWYRKKSGSTNEESISKGGRYVETINEGSKSFSLRINDLTVEDSGTYRCKLSWWTQNWRCSNSDVYGGGTKVEIK

SEQ ID NO: 59 - protein, 484 aa, artificial sequence
  soloMER D1-Fc-C4 Quad-X (NAR FW4)-Lead
ARVDQSPSSLSASVGDRVTITCVLRDSHCATSSTYWYRKKSGSTNEESISKGGRYVETVNSGSKSFTLTISSLQPEDFATYYCASECQYGLAEYDVYGGGTVVTVNGSGGGSGGGGSGEPKSSDKTHTCPPCPAPELLGGPSVFLFPPKPKDTLMISRTPEVTCVVVDVSHEDPEVKFNWYVDGVEVHNAKTKPREEQYNSTYRVVSVLTVLHQDWLNGKEYKCKVSNKALPAPIEKTISKAKGQPREPQVYTLPPSRDELTKNQVSLTCLVKGFYPSDIAVEWESNGQPENNYKTTPPVLDSDGSFFLYSKLTVDKSRWQQGNVFSCSVMHEALHNHYTQKSLSLSPGKGGGGSGGGGSGGGGSGGGGSGGGGSARVDQSPSSLSASVGDRVTITCVLRDSNCGLSSTYWYRKKSGSTNEESISKGGRYVETINEGSKSFSLRINDLTVEDSGTYRCKLSWWTQNWRCSNSDVYGGGTVVTVN

SEQ ID NO: 60 - protein, 483 aa, artificial sequence
  WT D1-Fc-C4 Quad-X
ARVDQTPQTITKETGESLTINCVLRDSHCATSSTYWYRKKSGSTNEESISKGGRYVETVNSGSKSFSLRINDLTVEDSGTYRCASECQYGLAEYDVYGGGTVVTVNGSGGGSGGGGSGEPKSSDKTHTCPPCPAPELLGGPSVFLFPPKPKDTLMISRTPEVTCVVVDVSHEDPEVKFNWYVDGVEVHNAKTKPREEQYNSTYRVVSVLTVLHQDWLNGKEYKCKVSNKALPAPIEKTISKAKGQPREPQVYTLPPSRDELTKNQVSLTCLVKGFYPSDIAVEWESNGQPENNYKTTPPVLDSDGSFFLYSKLTVDKSRWQQGNVFSCSVMHEALHNHYTQKSLSLSPGKGGGGSGGGGSGGGGSGGGGSGAHSARVDQTPQTITKETGESLTINCVLRDSNCGLSSTYWYRKKSGSTNEESISKGGRYVETINEGSKSFSLRINDLTVEDSGTYRCKLSWWTQNWRCSNSDVYGGGTVVTVN

SEQ ID NO: 61 - protein, 107 aa, artificial sequence
  P3A1
TRVDQTPRTATKETGESLTINCVLTDTSYGLYSTSWFRKNPGTTDWERMSIGGRYVESVNKGAKSFSLRIKDLTVADSATYYCKAREARHPWLRQWYDGAGTVLTVN

SEQ ID NO: 62 - protein, 107 aa, artificial sequence
  P3A1 V1
TRVDQSPSSLSASVGDRVTITCVLTDTSYGLYSTSWFRKNPGTTDWERMSIGGRYVESVNKGAKSFTLTISSLQPEDFATYYCKAREARHPWLRQWYDGAGTKVEIK

SEQ ID NO: 63 - protein, 107 aa, artificial sequence
  P3A1 V4
TRVDQSPSSLSASVGDRVTITCVLTDTSYGLYSTSWFQQKPGTTDWERMSIGGRYSGSGSKGAKSFTLTISSLQPEDFATYYCKAREARHPWLRQWYDGAGTKVEIK

SEQ ID NO: 64 - protein, 105 aa, artificial sequence
  E4WT
ASVNQTPRTATKETGESLTINCVLTDTKYLYSTSWFRKNPGTTDWERMSIGGRYVESVNKGAKSFSLRIKDLTVADSATYICRAWTSFEEQVKDVYGAGTVLTVN

SEQ ID NO: 65 - protein, 105 aa, artificial sequence
  E4V1
ASVNQSPSSLSASVGDRVTITCVLTDTKYLYSTSWFRKNPGTTDWERMSIGGRYVESVNKGAKSFSLRIKDLTVADSATYICRAWTSFEEQVKDVYGGGTKVEIK

SEQ ID NO: 66 - protein, 105 aa, artificial sequence
  E4V2
ASVNQSPSSLSASVGDRVTITCVLTDTKYLYSTSWFRKNPGTTDWERMSIGGRYVESVNKGAKSFTLTISSLQPEDFATYYCRAWTSFEEQVKDVYGGGTKVEIK

SEQ ID NO: 67 - protein, 105 aa, artificial sequence
  E4V3
ASVNQSPSSLSASVGDRVTITCVLTDTKYLYSTSWFRKNPGTTDWERMSIGGRFSGSGSKGAKSFTLTISSLQPEDFATYYCRAWTSFEEQVKDVYGGGTKVEIK

SEQ ID NO: 68 - protein, 105 aa, artificial sequence
  E4V4
ASVNQSPSSLSASVGDRVTITCVLTDTKYLYSTSWYQQKPGTTDWERMSIGGRYVESVNKGAKSFTLTISSLQPEDFATYYCRAWTSFEEQVKDVYGGGTKVEIK

SEQ ID NO: 69 - protein, 105 aa, artificial sequence
  E4V5
ASVNQSPSSLSASVGDRVTITCVLTDTKYLYSTSWYQQKPGTTDWERMSIGGRFSGSGSKGAKSFTLTISSLQPEDFATYYCRAWTSFEEQVKDVYGGGTKVEIK

SEQ ID NO: 70 - protein, 108 aa, artificial sequence
  78WT
TRVDQTPRTATKETGESLTINCVLTDTNYSLYATSWFRKNPGTTDWERMSIGGRYVESVNKGAKSFSLRIKDLTVADSATYICRAVWFPYFISDMWDVYGAGTVLTVN

SEQ ID NO: 71 - protein, 108 aa, artificial sequence
  78V1
TRVDQSPSSLSASVGDRVTITCVLTDTNYSLYATSWFRKNPGTTDWERMSIGGRYVESVNKGAKSFSLRIKDLTVADSATYICRAVWFPYFISHMWDVYGGGTKVEIK

SEQ ID NO: 72 - protein, 108 aa, artificial sequence
  78V2
TRVDQSPSSLSASVGDRVTITCVLTDTNYSLYATSWFRKNPGTTDWERMSIGGRYVESVNKGAKSFTLTISSLQPEDFATYYCRAVWFPYFISDMWDVYGGGTKVEIK

SEQ ID NO: 73 - protein, 108 aa, artificial sequence
  78V3
TRVDQSPSSLSASVGDRVTITCVLTDTNYSLYATSWYQQKPGKTDWERMSIGGRYVESVNKGAKSFTLTISSLQPEDFATYYCRAVWFPYFISDMWDVYGGGTKVEIK

SEQ ID NO: 74 - protein, 108 aa, artificial sequence
  78V4
TRVDQSPSSLSASVGDRVTITCVLTDTNYSLYATSWFRKNPGTTDWERMSIGGRFSGSGSKGAKSFTLTISSLQPEDFATYYCRAVWFPYFISDMWDVYGGGTKVEIK

SEQ ID NO: 75 - protein, 108 aa, artificial sequence
  78V5
TRVDQSPSSLSASVGDRVTITCVLTDTNYSLYATSWYQQKPGKTDWERMSIGGRFSGSGSKGAKSFTLTISSLQPEDFATYYCRAVWFPYFISDMWDVYGGGTKVEIK

SEQ ID NO: 76 - protein, 105 aa, artificial sequence
  E4V2B09
ASVNQSPSSLSASVGDRVTITCVLTGTGYWYSTSWFRKNPGTSNEDRIIIGGRYVESVNKGTKSFTLTISSLQPEDFATYYCRAWTSFEEQVKDVYGGGTKVEIK

SEQ ID NO: 77 - protein, 105 aa, artificial sequence
  E4V2D10
ASVNQSPSSLSASVGDRVTITCVLTGAGYWFATSWFRKNPGTSDKESISNSGRYVESVNKRSMSFTLTISSLQPEDFATYYCRAWTSFEEQVKDVYGGGTKVEIK

SEQ ID NO: 78 - protein, 105 aa, artificial sequence
  E4V2F3
ASVNQSPSSLSASVGDRVTITCVLTDTNYWYSTSWFRKNPGTTNEDRIIISGRYVESVNNGPKSFTLTISSLQPEDFATYYCRAWTSFEEQVKDVYGGGTKVEIK

SEQ ID NO: 79 - protein, 105 aa, artificial sequence
  E4V2Cc8
ASVNQSPSSLSASVGDRVTITCVLTSAGYLYATSWFRKNPGTSDKESMIIGRRYVESVNNRSMSFTLTISSLQPEDFATYYCRAWTSFEEQVKDVYGGGTKVEIK

SEQ ID NO: 80 - protein, 105 aa, artificial sequence
  E4V2Cc9
ASVNQSPSSLSASVGDRVTITCVLTGTEYLYSTSWFRKNPGTPNEDRMINGGRYVESVNKGTMSFTLTISSLQPEDFATYYCRAWTSFEEQVKDVYGGGTKVEIK

SEQ ID NO: 81 - protein, 105 aa, artificial sequence
  E4V2Ee6
ASVNQSPSSLSASVGDRVTITCVLTDTRYLYATSWFRKNPGTTNKESISNGGRYVESVNKRSMSFTLTISSLQPEDFATYYCRAWTSFEEQVKDVYGGGTKVEIK

SEQ ID NO: 82 - protein, 105 aa, artificial sequence
  E4V2Ee8
ASVNQSPSSLSASVGDRVTITCVLTGASYWYSTSWFRKNPGTTDEESMSNGGRYVESVNKRPMSFTLTISSLQPEDFATYYCRAWTSFEEQVKDVYGGGTKVEIK

SEQ ID NO: 83 - protein, 105 aa, artificial sequence
  E4V2Gg11
ASVNQSPSSLSASVGDRVTITCVLTGTRYWFSTSWFRKNPGTTDEDSISNGGRYVESVNNGSMSFTLTISSLQPEDFATYYCRAWTSFEEQVKDVYGGGTKVEIK

SEQ ID NO: 84 - protein, 112 aa, artificial sequence
  D3WT
ASVNQTPRTATKETGESLTINCVLTDTSYGLYSTSWFRKNPGTTDWERMSIGGRYVESVNKRAKSFSLRIKDLTVADSATYYCKAQSGMAISTGSGHGYNWYDGAGTVLTVN

SEQ ID NO: 85 - protein, 112 aa, artificial sequence
  D3WT V1
ASVNQSPSSLSASVGDRVTITCVLTDTSYGLYSTSWFRKNPGTTDWERMSIGGRYVESVNKRAKSFSLRIKDLTVADSATYYCKAQSGMAISTGSGHGYNWYDGAGTKVEIK

SEQ ID NO: 86 - protein, 112 aa, artificial sequence
  D3WT V2
ASVNQSPSSLSASVGDRVTITCVLTDTSYGLYSTSWFRKNPGTTDWERMSIGGRYVESVNKRAKSFTLTISSLQPEDFATYYCKAQSGMAISTGSGHGYNWYDGAGTKVEIK

SEQ ID NO: 87 - protein, 112 aa, artificial sequence
  D3WT V4
ASVNQSPSSLSASVGDRVTITCVLTDTSYGLYSTSWYQQKPGTTDWERMSIGGRYVESVNKRAKSFTLTISSLQPEDFATYYCKAQSGMAISTGSGHGYNWYDGAGTKVEIK

SEQ ID NO: 88 - protein, 112 aa, artificial sequence
  D3WT V5
ASVNQSPSSLSASVGDRVTITCVLTDTSYGLYSTSWYQQKPGTTDWERMSIGGRFSGSGSKRAKSFTLTISSLQPEDFATYYCKAQSGMAISTGSGHGYNWYDGAGTKVEIK

SEQ ID NO: 89 - protein, 25 aa, artificial sequence
  D3V2 FW1
ASVNQSPSSLSASVGDRVTITCVLT

SEQ ID NO: 90 - protein, 8 aa, artificial sequence
  D3V2 CDR1
DTSYGLYS

SEQ ID NO: 91 - protein, 10 aa, artificial sequence
  D3V2 FW2
TSWFRKNPGT

SEQ ID NO: 92 - protein, 9 aa, artificial sequence
  D3V2 HV2
TDWERMSIG

SEQ ID NO: 93 - protein, 8 aa, artificial sequence
  D3V2 FW3a
GRYVESVN

SEQ ID NO: 94 - protein, 5 aa, artificial sequence
  D3V2 HV4
KRAKS

SEQ ID NO: 95 - protein, 20 aa, artificial sequence
  D3V2 FW3b
FTLTISSLQPEDFATYYCKA

SEQ ID NO: 96 - protein, 17 aa, artificial sequence
  D3V2 CDR3
QSGMAISTGSGHGYNWY

SEQ ID NO: 97 - protein, 10 aa, artificial sequence
  D3V2 FW4
DGAGTKVEIK

SEQ ID NO: 98 - protein, 228 aa, artificial sequence
  D3 V2 PAN3 F11
ASVNQSPSSLSASVGDRVTITCVLTDTNYGLYATSWFRKNPGTSNEDRIIISGRYVESVNKRTKSFTLTISSLQPEDFATYYCKAQSGMAISTGSGHGYNWYDGAGTKVEIKQASGAAAAPSVFIFPPSDEQLKSGTASVVCLLNNFYPREAKVQWKVDNALQSGNSQESVTEQDSKDSTYSLSSTLTLSKADYEKHKVYACEVTHQGLSSPVTKSFNRGESHHHHHH

SEQ ID NO: 99 - protein, 228 aa, artificial sequence
  D3 V2 PAN3 E08
ASVNQSPSSLSASVGDRVTITCVLTDTRYGLYSTSWFRKNPGTTDKERISIGGRYVESVNKRTKSFTLTISSLQPEDFATYYCKAQSGMAISTGSGHGYNWYDGAGTKVEIKQASGAAAAPSVFIFPPSDEQLKSGTASVVCLLNNFYPREAKVQWKVDNALQSGNSQESVTEQDSKDSTYSLSSTLTLSKADYEKHKVYACEVTHQGLSSPVTKSFNRGESHHHHHH

SEQ ID NO: 100 - protein, 228 aa, artificial sequence
  D3 V2 PAN F01
ASVNQSPSSLSASVGDRVTITCVLTDTKYGLYSTSWFRKNPGTTDKERISIGGRYVESVNKRTKSFTLTISSLQPEDFATYYCKAQSGMAISTGSGHGYNWYDGAGTKVEIKQASGAAAAPSVFIFPPSDEQLKSGTASVVCLLNNFYPREAKVQWKVDNALQSGNSQESVTEQDSKDSTYSLSSTLTLSKADYEKHKVYACEVTHQGLSSPVTKSFNRGESHHHHHH

SEQ ID NO: 101 - protein, 228 aa, artificial sequence
  D3 V2 PAN G02
ASVNQSPSSLSASVGDRVTITCVLTDTNYGLYATSWFRKNPGTTDEERMSIGGRYVESVNKRSKSFTLTISSLQPEDFATYYCKAQSGMAISTGSGHGYNWYDGAGTKVEIKQASGAAAAPSVFIFPPSDEQLKSGTASVVCLLNNFYPREAKVQWKVDNALQSGNSQESVTEQDSKDSTYSLSSTLTLSKADYEKHKVYACEVTHQGLSSPVTKSFNRGESHHHHHH